European Patent Specification EP 4 096 717 B1, published December 11, 2024. Title: TREATMENT OF CANCER. Applicant: INNATE PHARMA. The sequence listing filed with the application follows.

SEQUENCE LISTING (16 sequences)

SEQ ID NO: 1 - protein, 510 aa, homo sapiens
MPLSLGAEMWGPEAWLLLLLLLASFTGRCPAGELETSDVVTVVLGQDAKLPCFYRGDSGEQVGQVAWARVDAGEGAQELALLHSKYGLHVSPAYEGRVEQPPPPRNPLDGSVLLRNAVQADEGEYECRVSTFPAGSFQARLRLRVLVPPLPSLNPGPALEEGQGLTLAASCTAEGSPAPSVTWDTEVKGTTSSRSFKHSRSAAVTSEFHLVPSRSMNGQPLTCVVSHPGLLQDQRITHILHVSFLAEASVRGLEDQNLWHIGREGAMLKCLSEGQPPPSYNWTRLDGPLPSGVRVDGDTLGFPPLTTEHSGIYVCHVSNEFSSRDSQVTVDVLDPQEDSGKQVDLVSASVVVVGVIAALLFCLLVVVVVLMSRYHRRKAQQMTQKYEEELTLTRENSIRRLHSHHTDPRSQPEESVGLRAEGHPDSLKDNSSCSVMSEEPEGRSYSTLTTVREIETQTELLSPGSGRAEEEEDQDEGIKQAMNHFVQENGTLRAKPTGNGIYINGRGHLV

SEQ ID NO: 2 - protein, 113 aa, homo sapiens
GELETSDVVTVVLGQDAKLPCFYRGDSGEQVGQVAWARVDAGEGAQELALLHSKYGLHVSPAYEGRVEQPPPPRNPLDGSVLLRNAVQADEGEYECRVSTFPAGSFQARLRLR

SEQ ID NO: 3 - protein, 117 aa, artificial
  synthetic
EVQLVESGGGLVQPGGSLRLSCAASGFTFSSYNMNWVRQAPGKGLEWVSYISSSSSTIYYADSVKGRFTISRDNAKNSLSLQMNSLRDEDTAVYYCARAYYYGMDVWGQGTTVTVSS

SEQ ID NO: 4 - protein, 111 aa, Artificial
  Synthetic
DIQMTQSPSSVSASVGDRVTITCRASQGISGWLAWYQQKPGKAPKFLIYAASTLQSGVPSRFSGSGSGTDFTLTISSLQPEDFATYYCQQANSFPPTFGGGTKVEIKRTVA

SEQ ID NO: 5 - protein, 447 aa, Artificial
  Synthetic
EVQLVESGGGLVQPGGSLRLSCAASGFTFSSYNMNWVRQAPGKGLEWVSYISSSSSTIYYADSVKGRFTISRDNAKNSLSLQMNSLRDEDTAVYYCARAYYYGMDVWGQGTTVTVSSASTKGPSVFPLAPSSKSTSGGTAALGCLVKDYFPEPVTVSWNSGALTSGVHTFPAVLQSSGLYSLSSVVTVPSSSLGTQTYICNVNHKPSNTKVDKRVEPKSCDKTHTCPPCPAPELLGGPSVFLFPPKPKDTLMISRTPEVTCVVVDVSHEDPEVKFNWYVDGVEVHNAKTKPREEQYNSTYRVVSVLTVLHQDWLNGKEYKCKVSNKALPAPIEKTISKAKGQPREPQVYTLPPSREEMTKNQVSLTCLVKGFYPSDIAVEWESNGQPENNYKTTPPVLDSDGSFFLYSKLTVDKSRWQQGNVFSCSVMHEALHNHYTQKSLSLSPGK

SEQ ID NO: 6 - protein, 214 aa, Artificial
  Synthetic
DIQMTQSPSSVSASVGDRVTITCRASQGISGWLAWYQQKPGKAPKFLIYAASTLQSGVPSRFSGSGSGTDFTLTISSLQPEDFATYYCQQANSFPPTFGGGTKVEIKRTVAAPSVFIFPPSDEQLKSGTASVVCLLNNFYPREAKVQWKVDNALQSGNSQESVTEQDSKDSTYSLSSTLTLSKADYEKHKVYACEVTHQGLSSPVTKSFNRGEC

SEQ ID NO: 7 - protein, 115 aa, mus musculus
EVLLQQSGPELVKPGASVKIPCKASGYTFTDYTMDWVKQSHGKSLEWIGDINPNNDVTMYNEKFKGRATLTVDKSSSTAYMEVRSLTSEDTAVYYCVRGRGFAYWGQGTLVTVSA

SEQ ID NO: 8 - protein, 111 aa, mus musculus
DIVLTQSPASLIVSLGQRATISCRASQSVSTSSNSYMHWYQQKPGQPPKLLIRFASNLESGVPARFSGSGSGTYFTLNIHPVEEEDSATYYCQHSWEIPYTFGGGTKLEIK

SEQ ID NO: 9 - protein, 116 aa, Mus musculus
QVQLKQSGPGLVQPSQSLSITCTVSGFSLTNYGVHWVRQSPGKGLEWLGVIWSGGSTDYNAAFISRLSISKDTSKSQVFFKMNSLQADDTAIYYCARELIHAMDNWGQGTSVTVSS

SEQ ID NO: 10 - protein, 106 aa, Mus musculus
DIQMTQSPASLSVSVGETVTITCRASENIYSNLAWYQQKQGNSPQLLVFAATNLADGVPSRFSGSGSGTQYSLKINSLQSEDFGTYYCQHFWGTPTFGGGTKLEIK

SEQ ID NO: 11 - protein, 90 aa, Homo sapiens
PPLPSLNPGPALEEGQGLTLAASCTAEGSPAPSVTWDTEVKGTTSSRSFKHSRSAAVTSEFHLVPSRSMNGQPLTCVVSHPGLLQDQRIT

SEQ ID NO: 12 - protein, 103 aa, Homo sapiens
ASVRGLEDQNLWHIGREGAMLKCLSEGQPPPSYNWTRLDGPLPSGVRVDGDTLGFPPLTTEHSGIYVCHVSNEFSSRDSQVTVDVLDPQEDSGKQVDLVSASV

SEQ ID NO: 13 - protein, 14 aa, Artificial
  Synthetic
GKPIPNPLLGLDST

SEQ ID NO: 14 - protein, 479 aa, Artificial
  Synthetic
GELETSDVVTVVLGQDAKLPCFYRGDSGEQVGQVAWARVDAGEGAQELALLHSKYGLHVSPAYEGRVEQPPPPRNPLDGSVLLRNAVQADEGEYECRVSTFPAGSFQARLRLRVLVPPLPSLNPGPALEEGQGLTLAASCTAEGSPAPSVTWDTEVKGTTSSRSFKHSRSAAVTSEFHLVPSRSMNGQPLTCVVSHPGLLQDQRITHILHVSFLAEASVRGLEDQNLWHIGREGAMLKCLSEGQPPPSYNWTRLDGPLPSGVRVDGDTLGFPPLTTEHSGIYVCHVSNEFSSRDSQVTVDVLDPQEDSGKQVDLVSASVVVVGVIAALLFCLLVVVVVLMSRYHRRKAQQMTQKYEEELTLTRENSIRRLHSHHTDPRSQPEESVGLRAEGHPDSLKDNSSCSVMSEEPEGRSYSTLTTVREIETQTELLSPGSGRAEEEEDQDEGIKQAMNHFVQENGTLRAKPTGNGIYINGRGHLV

SEQ ID NO: 15 - protein, 363 aa, Artificial
  Synthetic
PPLPSLNPGPALEEGQGLTLAASCTAEGSPAPSVTWDTEVKGTTSSRSFKHSRSAAVTSEFHLVPSRSMNGQPLTCVVSHPGLLQDQRITHILHVSFLAEASVRGLEDQNLWHIGREGAMLKCLSEGQPPPSYNWTRLDGPLPSGVRVDGDTLGFPPLTTEHSGIYVCHVSNEFSSRDSQVTVDVLDPQEDSGKQVDLVSASVVVVGVIAALLFCLLVVVVVLMSRYHRRKAQQMTQKYEEELTLTRENSIRRLHSHHTDPRSQPEESVGLRAEGHPDSLKDNSSCSVMSEEPEGRSYSTLTTVREIETQTELLSPGSGRAEEEEDQDEGIKQAMNHFVQENGTLRAKPTGNGIYINGRGHLV

SEQ ID NO: 16 - protein, 263 aa, Artificial
  Synthetic
ASVRGLEDQNLWHIGREGAMLKCLSEGQPPPSYNWTRLDGPLPSGVRVDGDTLGFPPLTTEHSGIYVCHVSNEFSSRDSQVTVDVLDPQEDSGKQVDLVSASVVVVGVIAALLFCLLVVVVVLMSRYHRRKAQQMTQKYEEELTLTRENSIRRLHSHHTDPRSQPEESVGLRAEGHPDSLKDNSSCSVMSEEPEGRSYSTLTTVREIETQTELLSPGSGRAEEEEDQDEGIKQAMNHFVQENGTLRAKPTGNGIYINGRGHLV